European Patent Application EP 4 361 251 A1, published May 1, 2024. Title: Deacetoxycephalosporin C Producing Strain for 7-ADCA Production with High Concentration and High Purity and Production Method Using the Same. Applicant: AMICOGEN, INC. The sequence listing filed with the application follows.

SEQUENCE LISTING (23 sequences)

SEQ ID NO: 1 - protein, 398 aa, synthetic construct
  REGION 1..398: note = CefD(D7) protein (Streptomyces clavuligerus)
MAVADWEEARGRMLLDPTVVNLNTGSGGPLPRSAFERVTGFRAHLAAEPMDFLLREVPALLWQARESLARLIGGDPLRLALATNVTAAVNLVASSLRLEAPGEILLSDDEYTPMRWCWERVARRHGLELRTFRLPELPSDPAEITAAAVAAMGPRTRLFFFSHVVSTTGLILPAAELCEEARARGITTVVDGAHAPGFLDLDLSRIPCDFYAGSGHKWLLAPTGVGFLHLAPGRLEELEPTQVSWAYEPPEGSGPPAARDRFGSTPGLRRLECEGTRDICPWLATPESIDFQAELGPGAIRARRRELTDHARRLLADRPGRTLLTPDSPELSGGMVAYRLPPGTDAAELRRGLWERFRIEAAVAEQPPGPVLRISANFYTTEEEIDRLADALDALTGE

SEQ ID NO: 2 - protein, 10 aa, synthetic construct
  REGION 1..10: note = PTS1 sequence of CefD1 (Acremonium chrysogenum)
SGQSAARPRL

SEQ ID NO: 3 - protein, 408 aa, synthetic construct
  REGION 1..408: note = D7px
MAVADWEEARGRMLLDPTVVNLNTGSGGPLPRSAFERVTGFRAHLAAEPMDFLLREVPALLWQARESLARLIGGDPLRLALATNVTAAVNLVASSLRLEAPGEILLSDDEYTPMRWCWERVARRHGLELRTFRLPELPSDPAEITAAAVAAMGPRTRLFFFSHVVSTTGLILPAAELCEEARARGITTVVDGAHAPGFLDLDLSRIPCDFYAGSGHKWLLAPTGVGFLHLAPGRLEELEPTQVSWAYEPPEGSGPPAARDRFGSTPGLRRLECEGTRDICPWLATPESIDFQAELGPGAIRARRRELTDHARRLLADRPGRTLLTPDSPELSGGMVAYRLPPGTDAAELRRGLWERFRIEAAVAEQPPGPVLRISANFYTTEEEIDRLADALDALTGESGQSAARPRL

SEQ ID NO: 4 - DNA, 1230 bp, synthetic construct
  misc_feature 1..1230: note = codon optimized D7px coding DNA
  source 1..1230: mol_type = other DNA
atggccgttgcggactgggaggaggcgcgcggccgcatgctcctggatcccaccgttgtcaatctaaacacggggtcgggaggcccgctccccaggtccgccttcgagagggtcacaggtttccgtgcccacctggccgcggagccgatggacttcctgcttcgcgaggtgcctgctcttctctggcaggccagggagagcctcgcccgcctgatcggtggcgatcccttgcggctcgccctggcgaccaatgtcacggcagccgtgaatctggtcgccagttcgctgcgtctcgaggcaccgggtgagattcttctgtcggacgacgaatacacacccatgagatggtgctgggagcgcgtggcccgtaggcatggcttggagctccgcacattccgcctgccagagctgccaagcgatccggctgaaatcactgcagccgcagttgctgcaatgggaccgcggacgcgactctttttcttctcccacgtcgtttcgaccacgggtctcatactccccgctgcggagctctgcgaagaggcccgagcccgtggcatcacgacggtcgtcgatggcgcccatgcccctggttttctggatctcgacctcagccgtatcccgtgcgacttttacgccggttccggtcataagtggctcctggcacccactggcgttggcttcctccacttggcgccgggccgcctagaggaactcgagcctacacaggtctcatgggcctacgagcctccagagggctcgggccctccggcggcgcgagaccggtttgggagtaccccgggcctgcggaggctcgagtgcgagggcacgcgagatatctgcccctggctcgccacccccgaaagtatcgacttccaagcagagctaggtcccggggctatccgtgcgcgtcgtcgcgagctgaccgaccatgcgcggcgcctgctcgccgaccgtcctgggaggaccctccttactcctgactcgccggagctctcaggcggaatggttgcttacaggttgccacccggcaccgacgcagccgagctgcgccgtggcctgtgggagcgatttcgcatcgaggccgccgtcgccgaacagccgccgggccccgtgctacgcatctccgcgaatttctataccaccgaggaggagattgatcgactcgccgacgccctcgacgcccttacgggagagtccggccagtcggcggctcggccaagactctaatga

SEQ ID NO: 5 - DNA, 414 bp, synthetic construct
  misc_feature 1..414: note = Codon optimized CefE of Mycobacteroides abscessus subsp.abscessus (NCBI:txid1185650)
  source 1..414: mol_type = other DNA
atgacggacatcggtgaaccggagcctggtcagtaccggatcggcccgcacacggacttcggcaccgtcacgatcctggaccgggagccgggagccggagggctgcaggtgtactccgagcagggcggctgggccgacgccccgtacgacccgtcggccctgacggtcaacatcggagacctgctcgagtactggtcggggggcaggtggccggcgggccgccaccgggtgctcccgccacaggcggacgctccggaggaagacctggtgtctctcatcttcttctacgaactcgaccacgacgccgtcgtgaccccgctcgaccccccggtcggaaagatcgccggccggccgccggtcatcggcggcgatttcatccgggagaggctggacgccataaccgtcggctgataa

SEQ ID NO: 6 - DNA, 1077 bp, synthetic construct
  misc_feature 1..1077: note = Codon optimized CefE of Sphingomonas dokdonensis(NCBI:txid344880)
  source 1..1077: mol_type = other DNA
atgcatcgcgcgggcggcagcgggctcgtccccagtggccgcatcgccggctattggcgatgcgagcggccctggcgcatgcagcgccgatcccgctgctcgaccaaggccctggtgatgctggacacccccctggcgaaggtgccgaccctcagtctcgcagaccaggcagtcgatcccgaccgcttcgccgccgacctgggcggttcgttcaggcggttcggcttcgccatcgtcgcggaccatggcatcccggacgacctcatcgcccgggcctgggcgcagaccgaggccctgttcgcccagccggacgccgacaagcggggctactacgtggaaggcgcgggcggggcccgcggctacaccccgttcaagaccgagatcgcgaaggacgccaagcacgtcgacctgaaggagttctggcacgtggggcgagagctgcccacgggccaccggtacgcgggtgagatggccccgaacatctggcccgcccagcccgatggcttcaaggagaccttcgtcgagctgttccgcgctttcgacacggcgggcgacaagctcctgagcgccatcgcccgggacctcgggctggcgccggactggttcgacctggcggtcaaggacggcaactccgtcctccgcctgctgcactaccccccgatcccgatggacgcggagggcgtccgcgcgggagcccatgaggacatcaacctgatcacccttctcctgggtgccgaggaggctggactggagctgctcgaccgcgacagcgggaattggctggccatcaagcccccggagggcgcgatggtagtgaacgtcggggacatgctgcagcggttgaccaaccacgtcctgccgtccaccacccaccgcgtcgtcaatccgcccccggagcgccgggcccactcccgctacagcatgcccttctttctgcacccggcccccgacttcctgatcaagaccctgccccagaccgtcacctcctccaacccgaaccggtaccccaccccgatcacggcgcacgactacctccatgagcggcttgtggagatcggtctcatcaagaagtgataa

SEQ ID NO: 7 - DNA, 38 bp, synthetic construct
  misc_feature 1..38: note = E3-F primer
  source 1..38: mol_type = other DNA
cgcttgagcagacatcaccatgacggacatcggtgaac

SEQ ID NO: 8 - DNA, 30 bp, synthetic construct
  misc_feature 1..30: note = E3-R primer
  source 1..30: mol_type = other DNA
gctaagcttttatcagccgacggttatggc

SEQ ID NO: 9 - DNA, 37 bp, synthetic construct
  misc_feature 1..37: note = E8-F primer
  source 1..37: mol_type = other DNA
cgcttgagcagacatcaccatgcatcgcgcgggcggc

SEQ ID NO: 10 - DNA, 29 bp, synthetic construct
  misc_feature 1..29: note = E8-R primer
  source 1..29: mol_type = other DNA
gctaagcttttatcacttcttgatgagac

SEQ ID NO: 11 - DNA, 38 bp, synthetic construct
  misc_feature 1..38: note = D7px-F primer
  source 1..38: mol_type = other DNA
cgcttgagcagacatcaccatggccgttgcggactggg

SEQ ID NO: 12 - DNA, 29 bp, synthetic construct
  misc_feature 1..29: note = D7px-R primer
  source 1..29: mol_type = other DNA
tatgaattctcattagagtcttggccgag

SEQ ID NO: 13 - DNA, 2315 bp, synthetic construct
  misc_feature 1..2315: note = PEP3 promoter
  source 1..2315: mol_type = other DNA
gcggccgcccttgtatctctacacacaggctcaaatcaataagaagaacggttcgtctttttcgtttatatcttgcatcgtcccaaagctattggcgggatattctgtttgcagttggctgacttgaagtaatctctgcagatctttcgacactgaaatacgtcgagcctgctccgcttggaagcggcgaggagcctcgtcctgtcacaactaccaacatggagtacgataagggccagttccgccagctcattaagagccagttcatgggcgttggcatgatggccgtcatgcatctgtacttcaagtacaccaacgctcttctgatccagtcgatcatccgctgaaggcgctttcgaatctggttaagatccacgtcttcgggaagccagcgactggtgacctccagcgtccctttaaggctgccaacagctttctcagccagggccagcccaagaccgacaaggcctccctccagaacgccgagaagaactggaggggtggtgtcaaggaggagtaagctccttattgaagtcggaggacggagcggtgtcaagaggatattcttcgactctgtattatagataagatgatgaggaattggaggtagcatagcttcatttggatttgctttccaggctgagactctagcttggagcatagagggtcctttggctttcaatattctcaagtatctcgagtttgaacttattccctgtgaaccttttattcaccaatgagcattggaatgaacatgaatctgaggactgcaatcgccatgaggttttcgaaatacatccggatgtcgaaggcttggggcacctgcgttggttgaatttagaacgtggcactattgatcatccgatagctctgcaaagggcgttgcacaatgcaagtcaaacgttgctagcagttccaggtggaatgttatgatgagcattgtattaaatcaggagatatagcatgatctctagttagctcaccacaaaagtcagacggcgtaaccaaaagtcacacaacacaagctgtaaggatttcggcacggctacggaagacggagaagccaccttcagtggactcgagtaccatttaattctatttgtgtttgatcgagacctaatacagcccctacaacgaccatcaaagtcgtatagctaccagtgaggaagtggactcaaatcgacttcagcaacatctcctggataaactttaagcctaaactatacagaataagataggtggagagcttataccgagctcccaaatctgtccagatcatggttgaccggtgcctggatcttcctatagaatcatccttattcgttgacctagctgattctggagtgacccagagggtcatgacttgagcctaaaatccgccgcctccaccatttgtagaaaaatgtgacgaactcgtgagctctgtacagtgaccggtgactctttctggcatgcggagagacggacggacgcagagagaagggctgagtaataagccactggccagacagctctggcggctctgaggtgcagtggatgattattaatccgggaccggccgcccctccgccccgaagtggaaaggctggtgtgcccctcgttgaccaagaatctattgcatcatcggagaatatggagcttcatcgaatcaccggcagtaagcgaaggagaatgtgaagccaggggtgtatagccgtcggcgaaatagcatgccattaacctaggtacagaagtccaattgcttccgatctggtaaaagattcacgagatagtaccttctccgaagtaggtagagcgagtacccggcgcgtaagctccctaattggcgaattcccatccggcatctgtagggcgtccaaatatcgtgcctctcctgctttgccaggtgtatgaaaccggaaaggccgctcaggagctggccagcggcgcagaccgggaacacaagctggcagtcgacccatccggtgctctgcactcgacctgctgaggtccctcagtccctggtaggcagctttgccccgtctgtccgcccggtgtgtcggcggggttgacaaggtcgttgcgtcagtccaacatttgttgccatattttcctgctttccccaccagctgctcttttcttttctctttcttttcccatcttcagtatattcatcttcccatatgcatccaagaacctttatttcccctaagtaagtactttgctacatccatactccatccttcccatcccttattcctttgaacctttcagttcgagctttcccacttcatcgcagcttgactaacagctaccccgcttgagcagacatcacc

SEQ ID NO: 14 - DNA, 39 bp, synthetic construct
  misc_feature 1..39: note = PEP3-F primer
  source 1..39: mol_type = other DNA
gcaactagtgcggccgcccttgtatctctacacacaggc

SEQ ID NO: 15 - DNA, 19 bp, synthetic construct
  misc_feature 1..19: note = PEP3-R primer
  source 1..19: mol_type = other DNA
ggtgatgtctgctcaagcg

SEQ ID NO: 16 - DNA, 16610 bp, synthetic construct
  misc_feature 1..16610: note = pB-HCXEP3 plasmid
  source 1..16610: mol_type = other DNA
gtggcacttttcggggaaatgtgcgcggaacccctatttgtttatttttctaaatacattcaaatatgtatccgctcatgagacaataaccctgataaatgcttcaataatattgaaaaaggaagagtatgagtattcaacatttccgtgtcgcccttattcccttttttgcggcattttgccttcctgtttttgctcacccagaaacgctggtgaaagtaaaagatgctgaagatcagttgggtgcacgagtgggttacatcgaactggatctcaacagcggtaagatccttgagagttttcgccccgaagaacgttttccaatgatgagcacttttaaagttctgctatgtggcgcggtattatcccgtattgacgccgggcaagagcaactcggtcgccgcatacactattctcagaatgacttggttgagtactcaccagtcacagaaaagcatcttacggatggcatgacagtaagagaattatgcagtgctgccataaccatgagtgataacactgcggccaacttacttctgacaacgatcggaggaccgaaggagctaaccgcttttttgcacaacatgggggatcatgtaactcgccttgatcgttgggaaccggagctgaatgaagccataccaaacgacgagcgtgacaccacgatgcctgtagcaatggcaacaacgttgcgcaaactattaactggcgaactacttactctagcttcccggcaacaattaatagactggatggaggcggataaagttgcaggaccacttctgcgctcggcccttccggctggctggtttattgctgataaatctggagccggtgagcgtgggtctcgcggtatcattgcagcactggggccagatggtaagccctcccgtatcgtagttatctacacgacggggagtcaggcaactatggatgaacgaaatagacagatcgctgagataggtgcctcactgattaagcattggtaactgtcagaccaagtttactcatatatactttagattgatttaaaacttcatttttaatttaaaaggatctaggtgaagatcctttttgataatctcatgaccaaaatcccttaacgtgagttttcgttccactgagcgtcagaccccgtagaaaagatcaaaggatcttcttgagatcctttttttctgcgcgtaatctgctgcttgcaaacaaaaaaaccaccgctaccagcggtggtttgtttgccggatcaagagctaccaactctttttccgaaggtaactggcttcagcagagcgcagataccaaatactgtccttctagtgtagccgtagttaggccaccacttcaagaactctgtagcaccgcctacatacctcgctctgctaatcctgttaccagtggctgctgccagtggcgataagtcgtgtcttaccgggttggactcaagacgatagttaccggataaggcgcagcggtcgggctgaacggggggttcgtgcacacagcccagcttggagcgaacgacctacaccgaactgagatacctacagcgtgagctatgagaaagcgccacgcttcccgaagggagaaaggcggacaggtatccggtaagcggcagggtcggaacaggagagcgcacgagggagcttccagggggaaacgcctggtatctttatagtcctgtcgggtttcgccacctctgacttgagcgtcgatttttgtgatgctcgtcaggggggcggagcctatggaaaaacgccagcaacgcggcctttttacggttcctggccttttgctggccttttgctcacatgttctttcctgcgttatcccctgattctgtggataaccgtattaccgcctttgagtgagctgataccgctcgccgcagccgaacgaccgagcgcagcgagtcagtgagcgaggaagcggaagagcgcccaatacgcaaaccgcctctccccgcgcgttggccgattcattaatgcagctggcacgacaggtttcccgactggaaagcgggcagtgagcgcaacgcaattaatgtgagttagctcactcattaggcaccccaggctttacactttatgcttccggctcgtatgttgtgtggaattgtgagcggataacaatttcacacaggaaacagctatgaccatgattacgccaagcgcgcaattaaccctcactaaagggaacaaaagctgggcaaagctgtttaaaccccgggtacaattaaccctcactaaagggaacaaaagctgggcaaagcttccttgtatctctacacacaggctcaaatcaataagaagaacggttcgtctttttcgtttatatcttgcatcgtcccaaagctattggcgggatattctgtttgcagttggctgacttgaagtaatctctgcagatctttcgacactgaaatacgtcgagcctgctccgcttggaagcggcgaggagcctcgtcctgtcacaactaccaacatggagtacgataagggccagttccgccagctcattaagagccagttcatgggcgttggcatgatggccgtcatgcatctgtacttcaagtacaccaacgctcttctgatccagtcgatcatccgctgaaggcgctttcgaatctggttaagatccacgtcttcgggaagccagcgactggtgacctccagcgtccctttaaggctgccaacagctttctcagccagggccagcccaagaccgacaaggcctccctccagaacgccgagaagaactggaggggtggtgtcaaggaggagtaagctccttattgaagtcggaggacggagcggtgtcaagaggatattcttcgactctgtattatagataagatgatgaggaattggaggtagcatagcttcatttggatttgctttccaggctgagactctagcttggagcatagagggtcctttggctttcaatattctcaagtatctcgagtttgaacttattccctgtgaaccttttattcaccaatgagcattggaatgaacatgaatctgaggactgcaatcgccatgaggttttcgaaatacatccggatgtcgaaggcttggggcacctgcgttggttgaatttagaacgtggcactattgatcatccgatagctctgcaaagggcgttgcacaatgcaagtcaaacgttgctagcagttccaggtggaatgttatgatgagcattgtattaaatcaggagatatagcatgatctctagttagctcaccacaaaagtcagacggcgtaaccaaaagtcacacaacacaagctgtaaggatttcggcacggctacggaagacggagaagccaccttcagtggactcgagtaccatttaattctatttgtgtttgatcgagacctaatacagcccctacaacgaccatcaaagtcgtatagctaccagtgaggaagtggactcaaatcgacttcagcaacatctcctggataaactttaagcctaaactatacagaataagataggtggagagcttataccgagctcccaaatctgtccagatcatggttgaccggtgcctggatcttcctatagaatcatccttattcgttgacctagctgattctggagtgacccagagggtcatgacttgagcctaaaatccgccgcctccaccatttgtagaaaaatgtgacgaactcgtgagctctgtacagtgaccggtgactctttctggcatgcggagagacggacggacgcagagagaagggctgagtaataagccactggccagacagctctggcggctctgaggtgcagtggatgattattaatccgggaccggccgcccctccgccccgaagtggaaaggctggtgtgcccctcgttgaccaagaatctattgcatcatcggagaatatggagcttcatcgaatcaccggcagtaagcgaaggagaatgtgaagccaggggtgtatagccgtcggcgaaatagcatgccattaacctaggtacagaagtccaattgcttccgatctggtaaaagattcacgagatagtaccttctccgaagtaggtagagcgagtacccggcgcgtaagctccctaattggcgaattcccatccggcatctgtagggcgtccaaatatcgtgcctctcctgctttgccaggtgtatgaaaccggaaaggccgctcaggagctggccagcggcgcagaccgggaacacaagctggcagtcgacccatccggtgctctgcactcgacctgctgaggtccctcagtccctggtaggcagctttgccccgtctgtccgcccggtgtgtcggcggggttgacaaggtcgttgcgtcagtccaacatttgttgccatattttcctgctttccccaccagctgctcttttcttttctctttcttttcccatcttcagtatattcatcttcccatatgcatccaagaacctttatttcccctaagtaagtactttgctacatccatactccatccttcccatcccttattcctttgaacctttcagttcgagctttcccacttcatcgcagcttgactaacagctaccccgcttgagcagacatcaccatggaaccgaccagcaccccgcaggctccgatcgctgcttataaaccgcgtagcaacgaaatcctgtgggatggttatggtgttccgcatatctatggtgttgacgctccgagcgctttttatggttatggctgggctcaggctcgtagccatggtgataacatcctgcgtctgtatggtgaagctcgtggtaaaggcgctgaatattggggtccggattacgaacagacgaccgtttggctgctgaccaacggtgttccggaacgtgctcagcagtggtatgctcagcagagcccggattttcgtgctaacctggatgcttttgctgctggtatcaacgcttatgctcagcagaacccggatgatatcagcccggaagttcgtcaggttctgccggttagcggtgctgatgttgttgctcatgctcatcgtctgatgaactttctgtatgttgctagcccgggtcgtaccctgggtgaaggtgatccgccggatctggctgatcagggtagcaacagctgggctgttgctccgggtaaaaccgctaacggtaacgctctgctgctgcagaaccctcatctgagctggaccaccgattattttacctattatgaagctcatctggttaccccggattttgaagtgtatggtgctacccagatcggtctgccggttatccgtgttgcttttaaccagcgtatgggtatcaccaacaccgttaacggtatggttggtgctaccaactatcgtctgaccctgcaggatggtggttatctgtatgatggtcaggttcgtccgtttgaacgtcgtcaggctagctatcgtctgcgtcaggctgatggtaccaccgttgataaaccgctggaaatccgttccagcgttcatggtccggtttttgaacgtgctgatggtaccgctgttgctgttcgtgttgctggtctggatcgtccgggtatgctggaacagacttttgatatgatcaccgctgatagctttgatgattatgaagctgctctggctcgtatgcaggttccgaccttgaacatcgtttatgctgatcgtgaaggtaccatcaactatagctttaacggtgttgctccgaaacgtgctgaaggtgacatcgctttttggcagggtctggttccgggtgatagcagccgttatctgtggaccgaaacccatccgctggatgatctgccgcgtgttaccaacccgccgggtggttttgttcagaacagcaacgatccgccgtggaccccgacctggccggttacctataccccgaaagattttccgagctatctggctccgcagaccccgcatagcctgcgtgctcagcagagcgttcgtctgatgagcgaaaacgatgatctgaccctggaacgttttatggctctgcagctgagccatcgtgctgttatggctgatcgtaccctgccggatctgatcccggctgctctgatcgatccggatccggaagttcaggctgctgctcgtctgctggctgcgtgggatcgtgaatttaccagcgatagccgtgctgctctgctgtttgaagaatgggctcgtctgtttgctggtcagaactttgctggtcaggctggctttgctaccccgtggagcctggataaaccggttagcaccccgtatggtctgcgtgatccgaaagctgctgttgatcagctgcgtaccgctatcgctaacaccaaacgtaaatatggtgctatcgatcgtccgtttggtgatgctagccgtatgatcctgaacgatgttaacgttccgggtgctgctggttatggtaacctgggtagctttcgtgtttttacctggagcgatccggatgaaaacggtgtgcgtaccccggttcatggtgaaacctgggttgctatgatcgaatttagcaccccggttcgtgcttatggtctgatgagctatggtaacagccgtcagccgggtaccacccattatagcgatcagatcgaacgtgttagccgtgctgattttcgtgaactgctgctgcgtcgtgaacaggttgaagctgctgttcaggaacgtaccccgtttaactttaaaccgtgaagtagatgccgaccgcgagatccacttaacgttactgaaatcatcaaacagcttgacgaatctggatataagatcgttggtgtcgatgtcagctccggagttgagacaaatggtgttcaggatctcgataagatacgttcatttgtccaagcagcaaagagtgccttctagtgatttaatagctccatgtcaacaagaataaaacgcgttttcgggtttacctcttccagatacagctcatctgcaatgcattaatgcattgactgcaacctagtaacgccttncaggctccggcgaagagaagaatagcttagcagagctattttcattttcgggagacgagatcaagcagatcaacggtcgtcaagagacctacgagactgaggaatccgctcttggctccacgcgactatatatttgtctctaattgtactttgacatgctcctcttctttactctgatagcttgactatgaaaattccgtcaccagcncctgggttcgcaaagataattgcatgtttcttccttgaactctcaagcctacaggacacacattcatcgtaggtataaacctcgaaatcanttcctactaagatggtatacaatagtaaccatgcatggttgcctagtgaatgctccgtaacacccaatacgccggccgaaacttttttacaactctcctatgagtcgtttacccagaatgcacaggtacacttgtttagaggtaatccttctttctagaagtcctcgtgtactgtgtaagcgcccactccacatctccactcgaccaattcgccctatagtgagtcgtattagtaaattaaccctcactaaagggaacaaaagctgggcaaagcttgaggccggacaaattcagcctgcaggctaaagtttctattacatgatatttgtcgtggacaagggcgtctggggtaaaaaggaatgtgggcagagagctctcggcttaaagaccggcttcggagttccagacccactcgaactgaaaacgatgattagagataagtagatctatttggacagtataagaatcctagtcggctagtatttctccacttttactttaaaattccccagagtaagggggcaggttcgtcgtcacgggtagcctcgtctcgaggcatcgcggatagcattatcttggggtatcacgagtaacttcatcgtggcattatcgataggtactgtaagtactgtaggaacttatccgggcatggatatgtataggtacatacgatgcactaaaagtggagaaatactagccgagtagagatcttataccatccgaatagatttactccttataatcaaggggcaacaatcagttgtgacgatgtcggctgtgggagtgcagtttaggggtcatcaaagcacaggaaaacgtgttgtatggatgcctatcgtcttgactattagaaaggaagaggggaaaaaccctcatcaggagcgattgtaagttcggccatagtaatgatattggccattaatggacgtgtgtatgtatacatacacggttcatttgccgcattcggaccaaaaccgctgctgccgcagacacagtgcttccatggcctcgaacaaccggttattcttctcttccatgtcctcgggacgaaggaaatttcggagccctaacagccgtaccggacttgcgttaacatggttgcgaagaactaaagactgatggggtcatgattggcagtgttgacacttcatgtcttgaacctagctagcagaaaaatgaatgctctatgtgacactggtagatctcaacgcatcatgttccacctttagtgtaaacacggcaagctgtccgcaacgtcggtaccaacgtttgaacacacaaccttctgccactccaggagtttagcccacggcttactggatgaaacgtaatctcccgctaccccctcaattccattggggtctagagtagtcggaagaacggctgtcgccttgcgctgcggttaaagcacccaccgtggtggctactgcttctcgggaggagaaatcctgggtactcgagcacttgcgctaggggatgaaacatccatggcatattggcgaaagcaatgcgccatgttcggcgcggcacatgacactcttgagaagccgtattcttcgcaaactttcctatttacattcagcctctaactataacacgatcggaaatgcctgaacgagcccgccctcatgtgcctagcgtcaaacaacgccaagcacacaacgcctcctgctattcttccctcttctcactgccatcactgggcgcaagctgcaatgtccttctcgaattcaagcgggcaaatcaagattgggaaaatgcgccatcttggtttggatcttgatgtctatccgcatcaaggtcttggtttggtcgtttatttagtagcaaaggcaaatcaaaacgtgcgcgccaagtgccagggtccagactccagactggagcatttagcctgaatatcgtctctagaatctggtgctattattcaggatatagtaactatgatctactcgggccatgttcggctcctccgcacggccaagttgtctgccggcgtctggaccggactcatggcttggcttctccagggatagcatggcattggcaaaactctccgccacgattcgagcatagctaccgcagccacgcggcattgtttccagattgagatatgtcactattagccggaatgcaaacatcgagctgacctgcgcaacatctccatgagttccgaagtcgacctccgaagcaatattggtctagtattacggatgatatagtggtccccggacccaatgagccgtgtgttttttaccgcctttgctctgaggattaacaagattcgtgcaattggggactgtgcggagtaactgggctggtttactgctttgccgacgaaagaaacgtataaacagccgactcgtccactgccactcgggacgatctcccaacccagacagcttcccagaacccatcttcaacaccctgacaccatgccccagttcgacatcctatgcaagactcctccgaaggtgctcgtccgccagttcgtggagcgattcgagcgcccctcgggcgaaaagatcgccttgtgtgccgctgagcttacctacctctgctggatgatcacccacaacggcaccgccatcaagcgggctacctttatgagttacaataccatcattagcaactccctctcgtttgacatcgtcaacaagtccctgcagttcaagtacaagacccaaaaggccaccatcctcgaggcctcgctgaagaagctgatccccgcatgggaattcactatcatcccctactatggtcagaagcatcagtctgacatcaccgacattgtaagcagtctccagctccagtttgagtcctccgaggaggccgataaaggcaactcccactccaagaagatgctcaaggctttgctgagtgaaggcgagtccatctgggaaataaccgaaaagatcttgaacagtttcgagtacaccagccgcttcacgaagaccaagacgctgtaccagttcctgttcctcgccacattcatcaattgcggacgcttcagtgatatcaagaacgtggacccgaagtcattcaagctggttcagaacaagtacctcggtgtcatcattcagtgcttggtcaccgagaccaagacatccgtcagccgtcacatctacttcttttccgcaagagggcgtatcgaccccctagtgtacctagacgaattcctgcgcaactcggagcccgtcctaaagcgcgtcaaccgtaccggcaactctagcagcaacaagcaggagtaccagctcttgaaggataacctcgtccgatcatacaacaaggcgctcaagaagaacgctccatacagcatctttgctatcaagaatgggccaaagtcacacatcggccgccacctcatgacctcgtttctgtcgatgaagggcctcactgagcttaccaacgttgttggcaactggtccgataagcgcgccagcgccgtggcgcggacgacttacactcatcagatcacagctatccctgaccactacttcgccttggtcagtcgctattacgcctacgacccaattagtaaagagatgatcgctctcaaggacgaaaccaaccccatcgaggagtggcaacacatcgagcagcttaaaggctccgccgagggctcgatccggtaccccgcctggaacggtatcatatcgcaggaggtcttggattacctgagcagttatatcaatcgccgcatatgataaggatccacttaacgttactgaaatcatcaaacagcttgacgaatctggatataagatcgttggtgtcgatgtcagctccggagttgagacaaatggtgttcaggatctcgataagatacgttcatttgtccaagcagcaaagagtgccttctagtgatttaatagctccatgtcaacaagaataaaacgcgttttcgggtttacctcttccagatacagctcatctgcaatgcattaatgcattgactgcaacctagtaacgccttncaggctccggcgaagagaagaatagcttagcagagctattttcattttcgggagacgagatcaagcagatcaacggtcgtcaagagacctacgagactgaggaatccgctcttggctccacgcgactatatatttgtctctaattgtactttgacatgctcctcttctttactctgatagcttgactatgaaaattccgtcaccagcncctgggttcgcaaagataattgcatgtttcttccttgaactctcaagcctacaggacacacattcatcgtaggtataaacctcgaaatcanttcctactaagatggtatacaatagtaaccatgcatggttgcctagtgaatgctccgtaacacccaatacgccggccgaaacttttttacaactctcctatgagtcgtttacccagaatgcacaggtacacttgtttagaggtaatccttctttctagaagtcctcgtgtactgtgtaagcgcccactccacatctccactcgaccaattcgccctatagtgagtcgtattaagcttcctgcagttcgaagttcctattctctagaaagtataggaacttcagagcgctttccttgtatctctacacacaggctcaaatcaataagaagaacggttcgtctttttcgtttatatcttgcatcgtcccaaagctattggcgggatattctgtttgcagttggctgacttgaagtaatctctgcagatctttcgacactgaaatacgtcgagcctgctccgcttggaagcggcgaggagcctcgtcctgtcacaactaccaacatggagtacgataagggccagttccgccagctcattaagagccagttcatgggcgttggcatgatggccgtcatgcatctgtacttcaagtacaccaacgctcttctgatccagtcgatcatccgctgaaggcgctttcgaatctggttaagatccacgtcttcgggaagccagcgactggtgacctccagcgtccctttaaggctgccaacagctttctcagccagggccagcccaagaccgacaaggcctccctccagaacgccgagaagaactggaggggtggtgtcaaggaggagtaagctccttattgaagtcggaggacggagcggtgtcaagaggatattcttcgactctgtattatagataagatgatgaggaattggaggtagcatagcttcatttggatttgctttccaggctgagactctagcttggagcatagagggtcctttggctttcaatattctcaagtatctcgagtttgaacttattccctgtgaaccttttattcaccaatgagcattggaatgaacatgaatctgaggactgcaatcgccatgaggttttcgaaatacatccggatgtcgaaggcttggggcacctgcgttggttgaatttagaacgtggcactattgatcatccgatagctctgcaaagggcgttgcacaatgcaagtcaaacgttgctagcagttccaggtggaatgttatgatgagcattgtattaaatcaggagatatagcatgatctctagttagctcaccacaaaagtcagacggcgtaaccaaaagtcacacaacacaagctgtaaggatttcggcacggctacggaagacggagaagccaccttcagtggactcgagtaccatttaattctatttgtgtttgatcgagacctaatacagcccctacaacgaccatcaaagtcgtatagctaccagtgaggaagtggactcaaatcgacttcagcaacatctcctggataaactttaagcctaaactatacagaataagataggtggagagcttataccgagctcccaaatctgtccagatcatggttgaccggtgcctggatcttcctatagaatcatccttattcgttgacctagctgattctggagtgacccagagggtcatgacttgagcctaaaatccgccgcctccaccatttgtagaaaaatgtgacgaactcgtgagctctgtacagtgaccggtgactctttctggcatgcggagagacggacggacgcagagagaagggctgagtaataagccactggccagacagctctggcggctctgaggtgcagtggatgattattaatccgggaccggccgcccctccgccccgaagtggaaaggctggtgtgcccctcgttgaccaagaatctattgcatcatcggagaatatggagcttcatcgaatcaccggcagtaagcgaaggagaatgtgaagccaggggtgtatagccgtcggcgaaatagcatgccattaacctaggtacagaagtccaattgcttccgatctggtaaaagattcacgagatagtaccttctccgaagtaggtagagcgagtacccggcgcgtaagctccctaattggcccatccggcatctgtagggcgtccaaatatcgtgcctctcctgctttgcccggtgtatgaaaccggaaaggccgctcaggagctggccagcggcgcagaccgggaacacaagctggcagtcgacccatccggtgctctgcactcgacctgctgaggtccctcagtccctggtaggcagctttgccccgtctgtccgcccggtgtgtcggcggggttgacaaggtcgttgcgtcagtccaacatttgttgccatattttcctgctctccccaccagctgctcttttcttttctctttcttttcccatcttcagtatattcatcttcccatccaagaacctttatttcccctaagtaagtactttgctacatccatactccatccttcccatcccttattcctttgaacctttcagttcgagctttcccacttcatcgcagcttgactaacagctaccccgcttgagcagacatcaccatgcctgaactcaccgcgacgtctgtcgagaagtttctgatcgaaaagttcgacagcgtctccgacctgatgcagctctcggagggcgaagaatctcgtgctttcagcttcgatgtaggagggcgtggatatgtcctgcgggtaaatagctgcgccgatggtttctacaaagatcgttatgtttatcggcactttgcatcggccgcgctcccgattccggaagtgcttgacattggggaattcagcgagagcctgacctattgcatctcccgccgtgcacagggtgtcacgttgcaagacctgcctgaaaccgaactgcccgctgttctgcagccggtcgcggaggccatggatgcgatcgctgcggccgatcttagccagacgagcgggttcggcccattcggaccgcaaggaatcggtcaatacactacatggcgtgatttcatatgcgcgattgctgatccccatgtgtatcactggcaaactgtgatggacgacaccgtcagtgcgtccgtcgcgcaggctctcgatgagctgatgctttgggccgaggactgccccgaagtccggcacctcgtgcacgcggatttcggctccaacaatgtcctgacggacaatggccgcataacagcggtcattgactggagcgaggcgatgttcggggattcccaatacgaggtcgccaacatcttcttctggaggccgtggttggcttgtatggagcagcagacgcgctacttcgagcggaggcatccggagcttgcaggatcgccgcggctccgggcgtatatgctccgcattggtcttgaccaactctatcagagcttggttgacggcaatttcgatgatgcagcttgggcgcagggtcgatgcgacgcaatcgtccgatccggagccgggactgtcgggcgtacacaaatcgcccgcagaagcgcggccgtctggaccgatggctgtgtagaagtactcgccgatagtggaaaccgacgccccagcactcgtccgagggcaaaggaatagagtagatgccgaccgcgggatccacttaacgttactgaaatcatcaaacagcttgacgaatctggatataagatcgttggtgtcgatgtcagctccggagttgagacaaatggtgttcaggatctcgataagatacgttcatttgtccaagcagcaaagagtgccttctagtgatttaatagctccatgtcaacaagaataaaacgcgttttcgggtttacctcttccagatacagctcatctgcaatgcattaatgcattgactgcaacctagtaacgccttncaggctccggcgaagagaagaatagcttagcagagctattttcattttcgggagacgagatcaagcagatcaacggtcgtcaagagacctacgagactgaggaatccgctcttggctccacgcgactatatatttgtctctaattgtactttgacatgctcctcttctttactctgatagcttgactatgaaaattccgtcaccagcncctgggttcgcaaagataattgcatgtttcttccttgaactctcaagcctacaggacacacattcatcgtaggtataaacctcgaaatcanttcctactaagatggtatacaatagtaaccatgcatggttgcctagtgaatgctccgtaacacccaatacgccggccgaaacttttttacaactctcctatgagtcgtttacccagaatgcacaggtacacttgtttagaggtaatccttctttctagaagtcctcgtgtactgtgtaagcgcccactccacatctccactcgacctgcagttcgaagttcctattctctagaaagtataggaacttcagagcgctttccaattcgccctatagtgagtcgtattacgcgcgctcactggccgtcgttttacaacgtcgtgactgggaaaaccctggcgttacccaacttaatcgccttgcagcacatccccctttcgccagctggcgtaatagcgaagaggcccgcaccgatcgcccttcccaacagttgcgcagcctgaatggcgaatgggacgcgccctgtagcggcgcattaagcgcggcgggtgtggtggttacgcgcagcgtgaccgctacacttgccagcgccctagcgcccgctcctttcgctttcttcccttcctttctcgccacgttcgccggctttccccgtcaagctctaaatcgggggctccctttagggttccgatttagtgctttacggcacctcgaccccaaaaaacttgattagggtgatggttcacgtagtgggccatcgccctgatagacggtttttcgccctttgacgttggagtccacgttctttaatagtggactcttgttccaaactggaacaacactcaaccctatctcggtctattcttttgatttataagggattttgccgatttcggcctattggttaaaaaatgagctgatttaacaaaaatttaacgcgaattttaacaaaatattaacgcttacaatttag

SEQ ID NO: 17 - DNA, 3717 bp, synthetic construct
  misc_feature 1..3717: note = pB-TtrpC
  source 1..3717: mol_type = other DNA
gtggcacttttcggggaaatgtgcgcggaacccctatttgtttatttttctaaatacattcaaatatgtatccgctcatgagacaataaccctgataaatgcttcaataatattgaaaaaggaagagtatgagtattcaacatttccgtgtcgcccttattcccttttttgcggcattttgccttcctgtttttgctcacccagaaacgctggtgaaagtaaaagatgctgaagatcagttgggtgcacgagtgggttacatcgaactggatctcaacagcggtaagatccttgagagttttcgccccgaagaacgttttccaatgatgagcacttttaaagttctgctatgtggcgcggtattatcccgtattgacgccgggcaagagcaactcggtcgccgcatacactattctcagaatgacttggttgagtactcaccagtcacagaaaagcatcttacggatggcatgacagtaagagaattatgcagtgctgccataaccatgagtgataacactgcggccaacttacttctgacaacgatcggaggaccgaaggagctaaccgcttttttgcacaacatgggggatcatgtaactcgccttgatcgttgggaaccggagctgaatgaagccataccaaacgacgagcgtgacaccacgatgcctgtagcaatggcaacaacgttgcgcaaactattaactggcgaactacttactctagcttcccggcaacaattaatagactggatggaggcggataaagttgcaggaccacttctgcgctcggcccttccggctggctggtttattgctgataaatctggagccggtgagcgtgggtctcgcggtatcattgcagcactggggccagatggtaagccctcccgtatcgtagttatctacacgacggggagtcaggcaactatggatgaacgaaatagacagatcgctgagataggtgcctcactgattaagcattggtaactgtcagaccaagtttactcatatatactttagattgatttaaaacttcatttttaatttaaaaggatctaggtgaagatcctttttgataatctcatgaccaaaatcccttaacgtgagttttcgttccactgagcgtcagaccccgtagaaaagatcaaaggatcttcttgagatcctttttttctgcgcgtaatctgctgcttgcaaacaaaaaaaccaccgctaccagcggtggtttgtttgccggatcaagagctaccaactctttttccgaaggtaactggcttcagcagagcgcagataccaaatactgtccttctagtgtagccgtagttaggccaccacttcaagaactctgtagcaccgcctacatacctcgctctgctaatcctgttaccagtggctgctgccagtggcgataagtcgtgtcttaccgggttggactcaagacgatagttaccggataaggcgcagcggtcgggctgaacggggggttcgtgcacacagcccagcttggagcgaacgacctacaccgaactgagatacctacagcgtgagctatgagaaagcgccacgcttcccgaagggagaaaggcggacaggtatccggtaagcggcagggtcggaacaggagagcgcacgagggagcttccagggggaaacgcctggtatctttatagtcctgtcgggtttcgccacctctgacttgagcgtcgatttttgtgatgctcgtcaggggggcggagcctatggaaaaacgccagcaacgcggcctttttacggttcctggccttttgctggccttttgctcacatgttctttcctgcgttatcccctgattctgtggataaccgtattaccgcctttgagtgagctgataccgctcgccgcagccgaacgaccgagcgcagcgagtcagtgagcgaggaagcggaagagcgcccaatacgcaaaccgcctctccccgcgcgttggccgattcattaatgcagctggcacgacaggtttcccgactggaaagcgggcagtgagcgcaacgcaattaatgtgagttagctcactcattaggcaccccaggctttacactttatgcttccggctcgtatgttgtgtggaattgtgagcggataacaatttcacacaggaaacagctatgaccatgattacgccaagcgcgcaattaaccctcactaaagggaacaaaagctggagctccaccgcggtggcggccgctctagaactagtggatcccccgggctgcaggaattcgatatcaagcttatcgataccgtcgacctcgagacttaacgttactgaaatcatcaaacagcttgacgaatctggatataagatcgttggtgtcgatgtcagctccggagttgagacaaatggtgttcaggatctcgataagatacgttcatttgtccaagcagcaaagagtgccttctagtgatttaatagctccatgtcaacaagaataaaacgcgttttcgggtttacctcttccagatacagctcatctgcaatgcattaatgcattgactgcaacctagtaacgcctttcaggctccggcgaagagaagaatagcttagcagagctattttcattttcgggagacgagatcaagcagatcaacggtcgtcaagagacctacgagactgaggaatccgctcttggctccacgcgactatatatttgtctctaattgtactttgacatgctcctcttctttactctgatagcttgactatgaaaattccgtcaccagcccctgggttcgcaaagataattgcatgtttcttccttgaactctcaagcctacaggacacacattcatcgtaggtataaacctcgaaatcagttcctactaagatggtatacaatagtaaccatgcatggttgcctagtgaatgctccgtaacacccaatacgccggccgaaacttttttacaactctcctatgagtcgtttacccagaatgcacaggtacacttgtttagaggtaatccttctttctagaagtcctcgtgtactgtgtaagcgcccactccacatctccactcgatggtacccaattcgccctatagtgagtcgtattacgcgcgctcactggccgtcgttttacaacgtcgtgactgggaaaaccctggcgttacccaacttaatcgccttgcagcacatccccctttcgccagctggcgtaatagcgaagaggcccgcaccgatcgcccttcccaacagttgcgcagcctgaatggcgaatgggacgcgccctgtagcggcgcattaagcgcggcgggtgtggtggttacgcgcagcgtgaccgctacacttgccagcgccctagcgcccgctcctttcgctttcttcccttcctttctcgccacgttcgccggctttccccgtcaagctctaaatcgggggctccctttagggttccgatttagtgctttacggcacctcgaccccaaaaaacttgattagggtgatggttcacgtagtgggccatcgccctgatagacggtttttcgccctttgacgttggagtccacgttctttaatagtggactcttgttccaaactggaacaacactcaaccctatctcggtctattcttttgatttataagggattttgccgatttcggcctattggttaaaaaatgagctgatttaacaaaaatttaacgcgaattttaacaaaatattaacgcttacaatttag

SEQ ID NO: 18 - DNA, 7232 bp, synthetic construct
  misc_feature 1..7232: note = pB-D7pxcast
  source 1..7232: mol_type = other DNA
gtggcacttttcggggaaatgtgcgcggaacccctatttgtttatttttctaaatacattcaaatatgtatccgctcatgagacaataaccctgataaatgcttcaataatattgaaaaaggaagagtatgagtattcaacatttccgtgtcgcccttattcccttttttgcggcattttgccttcctgtttttgctcacccagaaacgctggtgaaagtaaaagatgctgaagatcagttgggtgcacgagtgggttacatcgaactggatctcaacagcggtaagatccttgagagttttcgccccgaagaacgttttccaatgatgagcacttttaaagttctgctatgtggcgcggtattatcccgtattgacgccgggcaagagcaactcggtcgccgcatacactattctcagaatgacttggttgagtactcaccagtcacagaaaagcatcttacggatggcatgacagtaagagaattatgcagtgctgccataaccatgagtgataacactgcggccaacttacttctgacaacgatcggaggaccgaaggagctaaccgcttttttgcacaacatgggggatcatgtaactcgccttgatcgttgggaaccggagctgaatgaagccataccaaacgacgagcgtgacaccacgatgcctgtagcaatggcaacaacgttgcgcaaactattaactggcgaactacttactctagcttcccggcaacaattaatagactggatggaggcggataaagttgcaggaccacttctgcgctcggcccttccggctggctggtttattgctgataaatctggagccggtgagcgtgggtctcgcggtatcattgcagcactggggccagatggtaagccctcccgtatcgtagttatctacacgacggggagtcaggcaactatggatgaacgaaatagacagatcgctgagataggtgcctcactgattaagcattggtaactgtcagaccaagtttactcatatatactttagattgatttaaaacttcatttttaatttaaaaggatctaggtgaagatcctttttgataatctcatgaccaaaatcccttaacgtgagttttcgttccactgagcgtcagaccccgtagaaaagatcaaaggatcttcttgagatcctttttttctgcgcgtaatctgctgcttgcaaacaaaaaaaccaccgctaccagcggtggtttgtttgccggatcaagagctaccaactctttttccgaaggtaactggcttcagcagagcgcagataccaaatactgtccttctagtgtagccgtagttaggccaccacttcaagaactctgtagcaccgcctacatacctcgctctgctaatcctgttaccagtggctgctgccagtggcgataagtcgtgtcttaccgggttggactcaagacgatagttaccggataaggcgcagcggtcgggctgaacggggggttcgtgcacacagcccagcttggagcgaacgacctacaccgaactgagatacctacagcgtgagctatgagaaagcgccacgcttcccgaagggagaaaggcggacaggtatccggtaagcggcagggtcggaacaggagagcgcacgagggagcttccagggggaaacgcctggtatctttatagtcctgtcgggtttcgccacctctgacttgagcgtcgatttttgtgatgctcgtcaggggggcggagcctatggaaaaacgccagcaacgcggcctttttacggttcctggccttttgctggccttttgctcacatgttctttcctgcgttatcccctgattctgtggataaccgtattaccgcctttgagtgagctgataccgctcgccgcagccgaacgaccgagcgcagcgagtcagtgagcgaggaagcggaagagcgcccaatacgcaaaccgcctctccccgcgcgttggccgattcattaatgcagctggcacgacaggtttcccgactggaaagcgggcagtgagcgcaacgcaattaatgtgagttagctcactcattaggcaccccaggctttacactttatgcttccggctcgtatgttgtgtggaattgtgagcggataacaatttcacacaggaaacagctatgaccatgattacgccaagcgcgcaattaaccctcactaaagggaacaaaagctggagctccaccgcggtggcggccgctctagaactagtgcggccgcccttgtatctctacacacaggctcaaatcaataagaagaacggttcgtctttttcgtttatatcttgcatcgtcccaaagctattggcgggatattctgtttgcagttggctgacttgaagtaatctctgcagatctttcgacactgaaatacgtcgagcctgctccgcttggaagcggcgaggagcctcgtcctgtcacaactaccaacatggagtacgataagggccagttccgccagctcattaagagccagttcatgggcgttggcatgatggccgtcatgcatctgtacttcaagtacaccaacgctcttctgatccagtcgatcatccgctgaaggcgctttcgaatctggttaagatccacgtcttcgggaagccagcgactggtgacctccagcgtccctttaaggctgccaacagctttctcagccagggccagcccaagaccgacaaggcctccctccagaacgccgagaagaactggaggggtggtgtcaaggaggagtaagctccttattgaagtcggaggacggagcggtgtcaagaggatattcttcgactctgtattatagataagatgatgaggaattggaggtagcatagcttcatttggatttgctttccaggctgagactctagcttggagcatagagggtcctttggctttcaatattctcaagtatctcgagtttgaacttattccctgtgaaccttttattcaccaatgagcattggaatgaacatgaatctgaggactgcaatcgccatgaggttttcgaaatacatccggatgtcgaaggcttggggcacctgcgttggttgaatttagaacgtggcactattgatcatccgatagctctgcaaagggcgttgcacaatgcaagtcaaacgttgctagcagttccaggtggaatgttatgatgagcattgtattaaatcaggagatatagcatgatctctagttagctcaccacaaaagtcagacggcgtaaccaaaagtcacacaacacaagctgtaaggatttcggcacggctacggaagacggagaagccaccttcagtggactcgagtaccatttaattctatttgtgtttgatcgagacctaatacagcccctacaacgaccatcaaagtcgtatagctaccagtgaggaagtggactcaaatcgacttcagcaacatctcctggataaactttaagcctaaactatacagaataagataggtggagagcttataccgagctcccaaatctgtccagatcatggttgaccggtgcctggatcttcctatagaatcatccttattcgttgacctagctgattctggagtgacccagagggtcatgacttgagcctaaaatccgccgcctccaccatttgtagaaaaatgtgacgaactcgtgagctctgtacagtgaccggtgactctttctggcatgcggagagacggacggacgcagagagaagggctgagtaataagccactggccagacagctctggcggctctgaggtgcagtggatgattattaatccgggaccggccgcccctccgccccgaagtggaaaggctggtgtgcccctcgttgaccaagaatctattgcatcatcggagaatatggagcttcatcgaatcaccggcagtaagcgaaggagaatgtgaagccaggggtgtatagccgtcggcgaaatagcatgccattaacctaggtacagaagtccaattgcttccgatctggtaaaagattcacgagatagtaccttctccgaagtaggtagagcgagtacccggcgcgtaagctccctaattggcgaattcccatccggcatctgtagggcgtccaaatatcgtgcctctcctgctttgccaggtgtatgaaaccggaaaggccgctcaggagctggccagcggcgcagaccgggaacacaagctggcagtcgacccatccggtgctctgcactcgacctgctgaggtccctcagtccctggtaggcagctttgccccgtctgtccgcccggtgtgtcggcggggttgacaaggtcgttgcgtcagtccaacatttgttgccatattttcctgctttccccaccagctgctcttttcttttctctttcttttcccatcttcagtatattcatcttcccatatgcatccaagaacctttatttcccctaagtaagtactttgctacatccatactccatccttcccatcccttattcctttgaacctttcagttcgagctttcccacttcatcgcagcttgactaacagctaccccgcttgagcagacatcaccatggccgttgcggactgggaggaggcgcgcggccgcatgctcctggatcccaccgttgtcaatctaaacacggggtcgggaggcccgctccccaggtccgccttcgagagggtcacaggtttccgtgcccacctggccgcggagccgatggacttcctgcttcgcgaggtgcctgctcttctctggcaggccagggagagcctcgcccgcctgatcggtggcgatcccttgcggctcgccctggcgaccaatgtcacggcagccgtgaatctggtcgccagttcgctgcgtctcgaggcaccgggtgagattcttctgtcggacgacgaatacacacccatgagatggtgctgggagcgcgtggcccgtaggcatggcttggagctccgcacattccgcctgccagagctgccaagcgatccggctgaaatcactgcagccgcagttgctgcaatgggaccgcggacgcgactctttttcttctcccacgtcgtttcgaccacgggtctcatactccccgctgcggagctctgcgaagaggcccgagcccgtggcatcacgacggtcgtcgatggcgcccatgcccctggttttctggatctcgacctcagccgtatcccgtgcgacttttacgccggttccggtcataagtggctcctggcacccactggcgttggcttcctccacttggcgccgggccgcctagaggaactcgagcctacacaggtctcatgggcctacgagcctccagagggctcgggccctccggcggcgcgagaccggtttgggagtaccccgggcctgcggaggctcgagtgcgagggcacgcgagatatctgcccctggctcgccacccccgaaagtatcgacttccaagcagagctaggtcccggggctatccgtgcgcgtcgtcgcgagctgaccgaccatgcgcggcgcctgctcgccgaccgtcctgggaggaccctccttactcctgactcgccggagctctcaggcggaatggttgcttacaggttgccacccggcaccgacgcagccgagctgcgccgtggcctgtgggagcgatttcgcatcgaggccgccgtcgccgaacagccgccgggccccgtgctacgcatctccgcgaatttctataccaccgaggaggagattgatcgactcgccgacgccctcgacgcccttacgggagagtccggccagtcggcggctcggccaagactctaatgaaagcttatcgataccgtcgacctcgagacttaacgttactgaaatcatcaaacagcttgacgaatctggatataagatcgttggtgtcgatgtcagctccggagttgagacaaatggtgttcaggatctcgataagatacgttcatttgtccaagcagcaaagagtgccttctagtgatttaatagctccatgtcaacaagaataaaacgcgttttcgggtttacctcttccagatacagctcatctgcaatgcattaatgcattgactgcaacctagtaacgcctttcaggctccggcgaagagaagaatagcttagcagagctattttcattttcgggagacgagatcaagcagatcaacggtcgtcaagagacctacgagactgaggaatccgctcttggctccacgcgactatatatttgtctctaattgtactttgacatgctcctcttctttactctgatagcttgactatgaaaattccgtcaccagcccctgggttcgcaaagataattgcatgtttcttccttgaactctcaagcctacaggacacacattcatcgtaggtataaacctcgaaatcagttcctactaagatggtatacaatagtaaccatgcatggttgcctagtgaatgctccgtaacacccaatacgccggccgaaacttttttacaactctcctatgagtcgtttacccagaatgcacaggtacacttgtttagaggtaatccttctttctagaagtcctcgtgtactgtgtaagcgcccactccacatctccactcgatggtacccaattcgccctatagtgagtcgtattacgcgcgctcactggccgtcgttttacaacgtcgtgactgggaaaaccctggcgttacccaacttaatcgccttgcagcacatccccctttcgccagctggcgtaatagcgaagaggcccgcaccgatcgcccttcccaacagttgcgcagcctgaatggcgaatgggacgcgccctgtagcggcgcattaagcgcggcgggtgtggtggttacgcgcagcgtgaccgctacacttgccagcgccctagcgcccgctcctttcgctttcttcccttcctttctcgccacgttcgccggctttccccgtcaagctctaaatcgggggctccctttagggttccgatttagtgctttacggcacctcgaccccaaaaaacttgattagggtgatggttcacgtagtgggccatcgccctgatagacggtttttcgccctttgacgttggagtccacgttctttaatagtggactcttgttccaaactggaacaacactcaaccctatctcggtctattcttttgatttataagggattttgccgatttcggcctattggttaaaaaatgagctgatttaacaaaaatttaacgcgaattttaacaaaatattaacgcttacaatttag

SEQ ID NO: 19 - DNA, 20 bp, synthetic construct
  misc_feature 1..20: note = T3 primer
  source 1..20: mol_type = other DNA
aattaaccctcactaaaggg

SEQ ID NO: 20 - DNA, 21 bp, synthetic construct
  misc_feature 1..21: note = T7 primer
  source 1..21: mol_type = other DNA
taatacgactcactatagggc

SEQ ID NO: 21 - DNA, 11368 bp, synthetic construct
  misc_feature 1..11368: note = pB-HF
  source 1..11368: mol_type = other DNA
gtggcacttttcggggaaatgtgcgcggaacccctatttgtttatttttctaaatacattcaaatatgtatccgctcatgagacaataaccctgataaatgcttcaataatattgaaaaaggaagagtatgagtattcaacatttccgtgtcgcccttattcccttttttgcggcattttgccttcctgtttttgctcacccagaaacgctggtgaaagtaaaagatgctgaagatcagttgggtgcacgagtgggttacatcgaactggatctcaacagcggtaagatccttgagagttttcgccccgaagaacgttttccaatgatgagcacttttaaagttctgctatgtggcgcggtattatcccgtattgacgccgggcaagagcaactcggtcgccgcatacactattctcagaatgacttggttgagtactcaccagtcacagaaaagcatcttacggatggcatgacagtaagagaattatgcagtgctgccataaccatgagtgataacactgcggccaacttacttctgacaacgatcggaggaccgaaggagctaaccgcttttttgcacaacatgggggatcatgtaactcgccttgatcgttgggaaccggagctgaatgaagccataccaaacgacgagcgtgacaccacgatgcctgtagcaatggcaacaacgttgcgcaaactattaactggcgaactacttactctagcttcccggcaacaattaatagactggatggaggcggataaagttgcaggaccacttctgcgctcggcccttccggctggctggtttattgctgataaatctggagccggtgagcgtgggtctcgcggtatcattgcagcactggggccagatggtaagccctcccgtatcgtagttatctacacgacggggagtcaggcaactatggatgaacgaaatagacagatcgctgagataggtgcctcactgattaagcattggtaactgtcagaccaagtttactcatatatactttagattgatttaaaacttcatttttaatttaaaaggatctaggtgaagatcctttttgataatctcatgaccaaaatcccttaacgtgagttttcgttccactgagcgtcagaccccgtagaaaagatcaaaggatcttcttgagatcctttttttctgcgcgtaatctgctgcttgcaaacaaaaaaaccaccgctaccagcggtggtttgtttgccggatcaagagctaccaactctttttccgaaggtaactggcttcagcagagcgcagataccaaatactgtccttctagtgtagccgtagttaggccaccacttcaagaactctgtagcaccgcctacatacctcgctctgctaatcctgttaccagtggctgctgccagtggcgataagtcgtgtcttaccgggttggactcaagacgatagttaccggataaggcgcagcggtcgggctgaacggggggttcgtgcacacagcccagcttggagcgaacgacctacaccgaactgagatacctacagcgtgagctatgagaaagcgccacgcttcccgaagggagaaaggcggacaggtatccggtaagcggcagggtcggaacaggagagcgcacgagggagcttccagggggaaacgcctggtatctttatagtcctgtcgggtttcgccacctctgacttgagcgtcgatttttgtgatgctcgtcaggggggcggagcctatggaaaaacgccagcaacgcggcctttttacggttcctggccttttgctggccttttgctcacatgttctttcctgcgttatcccctgattctgtggataaccgtattaccgcctttgagtgagctgataccgctcgccgcagccgaacgaccgagcgcagcgagtcagtgagcgaggaagcggaagagcgcccaatacgcaaaccgcctctccccgcgcgttggccgattcattaatgcagctggcacgacaggtttcccgactggaaagcgggcagtgagcgcaacgcaattaatgtgagttagctcactcattaggcaccccaggctttacactttatgcttccggctcgtatgttgtgtggaattgtgagcggataacaatttcacacaggaaacagctatgaccatgattacgccaagcgcgcaattaaccctcactaaagggaacaaaagctgggcaaagctgtttaaaccccgggtacgtaaattaaccctcactaaagggaacaaaagctgggcaaagcttgaggccggacaaattcagcctgcaggctaaagtttctattacatgatatttgtcgtggacaagggcgtctggggtaaaaaggaatgtgggcagagagctctcggcttaaagaccggcttcggagttccagacccactcgaactgaaaacgatgattagagataagtagatctatttggacagtataagaatcctagtcggctagtatttctccacttttactttaaaattccccagagtaagggggcaggttcgtcgtcacgggtagcctcgtctcgaggcatcgcggatagcattatcttggggtatcacgagtaacttcatcgtggcattatcgataggtactgtaagtactgtaggaacttatccgggcatggatatgtataggtacatacgatgcactaaaagtggagaaatactagccgagtagagatcttataccatccgaatagatttactccttataatcaaggggcaacaatcagttgtgacgatgtcggctgtgggagtgcagtttaggggtcatcaaagcacaggaaaacgtgttgtatggatgcctatcgtcttgactattagaaaggaagaggggaaaaaccctcatcaggagcgattgtaagttcggccatagtaatgatattggccattaatggacgtgtgtatgtatacatacacggttcatttgccgcattcggaccaaaaccgctgctgccgcagacacagtgcttccatggcctcgaacaaccggttattcttctcttccatgtcctcgggacgaaggaaatttcggagccctaacagccgtaccggacttgcgttaacatggttgcgaagaactaaagactgatggggtcatgattggcagtgttgacacttcatgtcttgaacctagctagcagaaaaatgaatgctctatgtgacactggtagatctcaacgcatcatgttccacctttagtgtaaacacggcaagctgtccgcaacgtcggtaccaacgtttgaacacacaaccttctgccactccaggagtttagcccacggcttactggatgaaacgtaatctcccgctaccccctcaattccattggggtctagagtagtcggaagaacggctgtcgccttgcgctgcggttaaagcacccaccgtggtggctactgcttctcgggaggagaaatcctgggtactcgagcacttgcgctaggggatgaaacatccatggcatattggcgaaagcaatgcgccatgttcggcgcggcacatgacactcttgagaagccgtattcttcgcaaactttcctatttacattcagcctctaactataacacgatcggaaatgcctgaacgagcccgccctcatgtgcctagcgtcaaacaacgccaagcacacaacgcctcctgctattcttccctcttctcactgccatcactgggcgcaagctgcaatgtccttctcgaattcaagcgggcaaatcaagattgggaaaatgcgccatcttggtttggatcttgatgtctatccgcatcaaggtcttggtttggtcgtttatttagtagcaaaggcaaatcaaaacgtgcgcgccaagtgccagggtccagactccagactggagcatttagcctgaatatcgtctctagaatctggtgctattattcaggatatagtaactatgatctactcgggccatgttcggctcctccgcacggccaagttgtctgccggcgtctggaccggactcatggcttggcttctccagggatagcatggcattggcaaaactctccgccacgattcgagcatagctaccgcagccacgcggcattgtttccagattgagatatgtcactattagccggaatgcaaacatcgagctgacctgcgcaacatctccatgagttccgaagtcgacctccgaagcaatattggtctagtattacggatgatatagtggtccccggacccaatgagccgtgtgttttttaccgcctttgctctgaggattaacaagattcgtgcaattggggactgtgcggagtaactgggctggtttactgctttgccgacgaaagaaacgtataaacagccgactcgtccactgccactcgggacgatctcccaacccagacagcttcccagaacccatcttcaacaccctgacaccatgccccagttcgacatcctatgcaagactcctccgaaggtgctcgtccgccagttcgtggagcgattcgagcgcccctcgggcgaaaagatcgccttgtgtgccgctgagcttacctacctctgctggatgatcacccacaacggcaccgccatcaagcgggctacctttatgagttacaataccatcattagcaactccctctcgtttgacatcgtcaacaagtccctgcagttcaagtacaagacccaaaaggccaccatcctcgaggcctcgctgaagaagctgatccccgcatgggaattcactatcatcccctactatggtcagaagcatcagtctgacatcaccgacattgtaagcagtctccagctccagtttgagtcctccgaggaggccgataaaggcaactcccactccaagaagatgctcaaggctttgctgagtgaaggcgagtccatctgggaaataaccgaaaagatcttgaacagtttcgagtacaccagccgcttcacgaagaccaagacgctgtaccagttcctgttcctcgccacattcatcaattgcggacgcttcagtgatatcaagaacgtggacccgaagtcattcaagctggttcagaacaagtacctcggtgtcatcattcagtgcttggtcaccgagaccaagacatccgtcagccgtcacatctacttcttttccgcaagagggcgtatcgaccccctagtgtacctagacgaattcctgcgcaactcggagcccgtcctaaagcgcgtcaaccgtaccggcaactctagcagcaacaagcaggagtaccagctcttgaaggataacctcgtccgatcatacaacaaggcgctcaagaagaacgctccatacagcatctttgctatcaagaatgggccaaagtcacacatcggccgccacctcatgacctcgtttctgtcgatgaagggcctcactgagcttaccaacgttgttggcaactggtccgataagcgcgccagcgccgtggcgcggacgacttacactcatcagatcacagctatccctgaccactacttcgccttggtcagtcgctattacgcctacgacccaattagtaaagagatgatcgctctcaaggacgaaaccaaccccatcgaggagtggcaacacatcgagcagcttaaaggctccgccgagggctcgatccggtaccccgcctggaacggtatcatatcgcaggaggtcttggattacctgagcagttatatcaatcgccgcatatgataaggatccacttaacgttactgaaatcatcaaacagcttgacgaatctggatataagatcgttggtgtcgatgtcagctccggagttgagacaaatggtgttcaggatctcgataagatacgttcatttgtccaagcagcaaagagtgccttctagtgatttaatagctccatgtcaacaagaataaaacgcgttttcgggtttacctcttccagatacagctcatctgcaatgcattaatgcattgactgcaacctagtaacgccttncaggctccggcgaagagaagaatagcttagcagagctattttcattttcgggagacgagatcaagcagatcaacggtcgtcaagagacctacgagactgaggaatccgctcttggctccacgcgactatatatttgtctctaattgtactttgacatgctcctcttctttactctgatagcttgactatgaaaattccgtcaccagcncctgggttcgcaaagataattgcatgtttcttccttgaactctcaagcctacaggacacacattcatcgtaggtataaacctcgaaatcanttcctactaagatggtatacaatagtaaccatgcatggttgcctagtgaatgctccgtaacacccaatacgccggccgaaacttttttacaactctcctatgagtcgtttacccagaatgcacaggtacacttgtttagaggtaatccttctttctagaagtcctcgtgtactgtgtaagcgcccactccacatctccactcgaccaattcgccctatagtgagtcgtattaagcttcctgcagttcgaagttcctattctctagaaagtataggaacttcagagcgctttccttgtatctctacacacaggctcaaatcaataagaagaacggttcgtctttttcgtttatatcttgcatcgtcccaaagctattggcgggatattctgtttgcagttggctgacttgaagtaatctctgcagatctttcgacactgaaatacgtcgagcctgctccgcttggaagcggcgaggagcctcgtcctgtcacaactaccaacatggagtacgataagggccagttccgccagctcattaagagccagttcatgggcgttggcatgatggccgtcatgcatctgtacttcaagtacaccaacgctcttctgatccagtcgatcatccgctgaaggcgctttcgaatctggttaagatccacgtcttcgggaagccagcgactggtgacctccagcgtccctttaaggctgccaacagctttctcagccagggccagcccaagaccgacaaggcctccctccagaacgccgagaagaactggaggggtggtgtcaaggaggagtaagctccttattgaagtcggaggacggagcggtgtcaagaggatattcttcgactctgtattatagataagatgatgaggaattggaggtagcatagcttcatttggatttgctttccaggctgagactctagcttggagcatagagggtcctttggctttcaatattctcaagtatctcgagtttgaacttattccctgtgaaccttttattcaccaatgagcattggaatgaacatgaatctgaggactgcaatcgccatgaggttttcgaaatacatccggatgtcgaaggcttggggcacctgcgttggttgaatttagaacgtggcactattgatcatccgatagctctgcaaagggcgttgcacaatgcaagtcaaacgttgctagcagttccaggtggaatgttatgatgagcattgtattaaatcaggagatatagcatgatctctagttagctcaccacaaaagtcagacggcgtaaccaaaagtcacacaacacaagctgtaaggatttcggcacggctacggaagacggagaagccaccttcagtggactcgagtaccatttaattctatttgtgtttgatcgagacctaatacagcccctacaacgaccatcaaagtcgtatagctaccagtgaggaagtggactcaaatcgacttcagcaacatctcctggataaactttaagcctaaactatacagaataagataggtggagagcttataccgagctcccaaatctgtccagatcatggttgaccggtgcctggatcttcctatagaatcatccttattcgttgacctagctgattctggagtgacccagagggtcatgacttgagcctaaaatccgccgcctccaccatttgtagaaaaatgtgacgaactcgtgagctctgtacagtgaccggtgactctttctggcatgcggagagacggacggacgcagagagaagggctgagtaataagccactggccagacagctctggcggctctgaggtgcagtggatgattattaatccgggaccggccgcccctccgccccgaagtggaaaggctggtgtgcccctcgttgaccaagaatctattgcatcatcggagaatatggagcttcatcgaatcaccggcagtaagcgaaggagaatgtgaagccaggggtgtatagccgtcggcgaaatagcatgccattaacctaggtacagaagtccaattgcttccgatctggtaaaagattcacgagatagtaccttctccgaagtaggtagagcgagtacccggcgcgtaagctccctaattggcccatccggcatctgtagggcgtccaaatatcgtgcctctcctgctttgcccggtgtatgaaaccggaaaggccgctcaggagctggccagcggcgcagaccgggaacacaagctggcagtcgacccatccggtgctctgcactcgacctgctgaggtccctcagtccctggtaggcagctttgccccgtctgtccgcccggtgtgtcggcggggttgacaaggtcgttgcgtcagtccaacatttgttgccatattttcctgctctccccaccagctgctcttttcttttctctttcttttcccatcttcagtatattcatcttcccatccaagaacctttatttcccctaagtaagtactttgctacatccatactccatccttcccatcccttattcctttgaacctttcagttcgagctttcccacttcatcgcagcttgactaacagctaccccgcttgagcagacatcaccatgcctgaactcaccgcgacgtctgtcgagaagtttctgatcgaaaagttcgacagcgtctccgacctgatgcagctctcggagggcgaagaatctcgtgctttcagcttcgatgtaggagggcgtggatatgtcctgcgggtaaatagctgcgccgatggtttctacaaagatcgttatgtttatcggcactttgcatcggccgcgctcccgattccggaagtgcttgacattggggaattcagcgagagcctgacctattgcatctcccgccgtgcacagggtgtcacgttgcaagacctgcctgaaaccgaactgcccgctgttctgcagccggtcgcggaggccatggatgcgatcgctgcggccgatcttagccagacgagcgggttcggcccattcggaccgcaaggaatcggtcaatacactacatggcgtgatttcatatgcgcgattgctgatccccatgtgtatcactggcaaactgtgatggacgacaccgtcagtgcgtccgtcgcgcaggctctcgatgagctgatgctttgggccgaggactgccccgaagtccggcacctcgtgcacgcggatttcggctccaacaatgtcctgacggacaatggccgcataacagcggtcattgactggagcgaggcgatgttcggggattcccaatacgaggtcgccaacatcttcttctggaggccgtggttggcttgtatggagcagcagacgcgctacttcgagcggaggcatccggagcttgcaggatcgccgcggctccgggcgtatatgctccgcattggtcttgaccaactctatcagagcttggttgacggcaatttcgatgatgcagcttgggcgcagggtcgatgcgacgcaatcgtccgatccggagccgggactgtcgggcgtacacaaatcgcccgcagaagcgcggccgtctggaccgatggctgtgtagaagtactcgccgatagtggaaaccgacgccccagcactcgtccgagggcaaaggaatagagtagatgccgaccgcgggatccacttaacgttactgaaatcatcaaacagcttgacgaatctggatataagatcgttggtgtcgatgtcagctccggagttgagacaaatggtgttcaggatctcgataagatacgttcatttgtccaagcagcaaagagtgccttctagtgatttaatagctccatgtcaacaagaataaaacgcgttttcgggtttacctcttccagatacagctcatctgcaatgcattaatgcattgactgcaacctagtaacgccttncaggctccggcgaagagaagaatagcttagcagagctattttcattttcgggagacgagatcaagcagatcaacggtcgtcaagagacctacgagactgaggaatccgctcttggctccacgcgactatatatttgtctctaattgtactttgacatgctcctcttctttactctgatagcttgactatgaaaattccgtcaccagcncctgggttcgcaaagataattgcatgtttcttccttgaactctcaagcctacaggacacacattcatcgtaggtataaacctcgaaatcanttcctactaagatggtatacaatagtaaccatgcatggttgcctagtgaatgctccgtaacacccaatacgccggccgaaacttttttacaactctcctatgagtcgtttacccagaatgcacaggtacacttgtttagaggtaatccttctttctagaagtcctcgtgtactgtgtaagcgcccactccacatctccactcgacctgcagttcgaagttcctattctctagaaagtataggaacttcagagcgctttccaattcgccctatagtgagtcgtattacgcgcgctcactggccgtcgttttacaacgtcgtgactgggaaaaccctggcgttacccaacttaatcgccttgcagcacatccccctttcgccagctggcgtaatagcgaagaggcccgcaccgatcgcccttcccaacagttgcgcagcctgaatggcgaatgggacgcgccctgtagcggcgcattaagcgcggcgggtgtggtggttacgcgcagcgtgaccgctacacttgccagcgccctagcgcccgctcctttcgctttcttcccttcctttctcgccacgttcgccggctttccccgtcaagctctaaatcgggggctccctttagggttccgatttagtgctttacggcacctcgaccccaaaaaacttgattagggtgatggttcacgtagtgggccatcgccctgatagacggtttttcgccctttgacgttggagtccacgttctttaatagtggactcttgttccaaactggaacaacactcaaccctatctcggtctattcttttgatttataagggattttgccgatttcggcctattggttaaaaaatgagctgatttaacaaaaatttaacgcgaattttaacaaaatattaacgcttacaatttag

SEQ ID NO: 22 - DNA, 15805 bp, synthetic construct
  misc_feature 1..15805: note = pB-HFD7px
  source 1..15805: mol_type = other DNA
gtggcacttttcggggaaatgtgcgcggaacccctatttgtttatttttctaaatacattcaaatatgtatccgctcatgagacaataaccctgataaatgcttcaataatattgaaaaaggaagagtatgagtattcaacatttccgtgtcgcccttattcccttttttgcggcattttgccttcctgtttttgctcacccagaaacgctggtgaaagtaaaagatgctgaagatcagttgggtgcacgagtgggttacatcgaactggatctcaacagcggtaagatccttgagagttttcgccccgaagaacgttttccaatgatgagcacttttaaagttctgctatgtggcgcggtattatcccgtattgacgccgggcaagagcaactcggtcgccgcatacactattctcagaatgacttggttgagtactcaccagtcacagaaaagcatcttacggatggcatgacagtaagagaattatgcagtgctgccataaccatgagtgataacactgcggccaacttacttctgacaacgatcggaggaccgaaggagctaaccgcttttttgcacaacatgggggatcatgtaactcgccttgatcgttgggaaccggagctgaatgaagccataccaaacgacgagcgtgacaccacgatgcctgtagcaatggcaacaacgttgcgcaaactattaactggcgaactacttactctagcttcccggcaacaattaatagactggatggaggcggataaagttgcaggaccacttctgcgctcggcccttccggctggctggtttattgctgataaatctggagccggtgagcgtgggtctcgcggtatcattgcagcactggggccagatggtaagccctcccgtatcgtagttatctacacgacggggagtcaggcaactatggatgaacgaaatagacagatcgctgagataggtgcctcactgattaagcattggtaactgtcagaccaagtttactcatatatactttagattgatttaaaacttcatttttaatttaaaaggatctaggtgaagatcctttttgataatctcatgaccaaaatcccttaacgtgagttttcgttccactgagcgtcagaccccgtagaaaagatcaaaggatcttcttgagatcctttttttctgcgcgtaatctgctgcttgcaaacaaaaaaaccaccgctaccagcggtggtttgtttgccggatcaagagctaccaactctttttccgaaggtaactggcttcagcagagcgcagataccaaatactgtccttctagtgtagccgtagttaggccaccacttcaagaactctgtagcaccgcctacatacctcgctctgctaatcctgttaccagtggctgctgccagtggcgataagtcgtgtcttaccgggttggactcaagacgatagttaccggataaggcgcagcggtcgggctgaacggggggttcgtgcacacagcccagcttggagcgaacgacctacaccgaactgagatacctacagcgtgagctatgagaaagcgccacgcttcccgaagggagaaaggcggacaggtatccggtaagcggcagggtcggaacaggagagcgcacgagggagcttccagggggaaacgcctggtatctttatagtcctgtcgggtttcgccacctctgacttgagcgtcgatttttgtgatgctcgtcaggggggcggagcctatggaaaaacgccagcaacgcggcctttttacggttcctggccttttgctggccttttgctcacatgttctttcctgcgttatcccctgattctgtggataaccgtattaccgcctttgagtgagctgataccgctcgccgcagccgaacgaccgagcgcagcgagtcagtgagcgaggaagcggaagagcgcccaatacgcaaaccgcctctccccgcgcgttggccgattcattaatgcagctggcacgacaggtttcccgactggaaagcgggcagtgagcgcaacgcaattaatgtgagttagctcactcattaggcaccccaggctttacactttatgcttccggctcgtatgttgtgtggaattgtgagcggataacaatttcacacaggaaacagctatgaccatgattacgccaagcgcgcaattaaccctcactaaagggaacaaaagctgggcaaagctgtttaattaaccctcactaaagggaacaaaagctggagctccaccgcggtggcggccgctctagaactagtgcggccgcccttgtatctctacacacaggctcaaatcaataagaagaacggttcgtctttttcgtttatatcttgcatcgtcccaaagctattggcgggatattctgtttgcagttggctgacttgaagtaatctctgcagatctttcgacactgaaatacgtcgagcctgctccgcttggaagcggcgaggagcctcgtcctgtcacaactaccaacatggagtacgataagggccagttccgccagctcattaagagccagttcatgggcgttggcatgatggccgtcatgcatctgtacttcaagtacaccaacgctcttctgatccagtcgatcatccgctgaaggcgctttcgaatctggttaagatccacgtcttcgggaagccagcgactggtgacctccagcgtccctttaaggctgccaacagctttctcagccagggccagcccaagaccgacaaggcctccctccagaacgccgagaagaactggaggggtggtgtcaaggaggagtaagctccttattgaagtcggaggacggagcggtgtcaagaggatattcttcgactctgtattatagataagatgatgaggaattggaggtagcatagcttcatttggatttgctttccaggctgagactctagcttggagcatagagggtcctttggctttcaatattctcaagtatctcgagtttgaacttattccctgtgaaccttttattcaccaatgagcattggaatgaacatgaatctgaggactgcaatcgccatgaggttttcgaaatacatccggatgtcgaaggcttggggcacctgcgttggttgaatttagaacgtggcactattgatcatccgatagctctgcaaagggcgttgcacaatgcaagtcaaacgttgctagcagttccaggtggaatgttatgatgagcattgtattaaatcaggagatatagcatgatctctagttagctcaccacaaaagtcagacggcgtaaccaaaagtcacacaacacaagctgtaaggatttcggcacggctacggaagacggagaagccaccttcagtggactcgagtaccatttaattctatttgtgtttgatcgagacctaatacagcccctacaacgaccatcaaagtcgtatagctaccagtgaggaagtggactcaaatcgacttcagcaacatctcctggataaactttaagcctaaactatacagaataagataggtggagagcttataccgagctcccaaatctgtccagatcatggttgaccggtgcctggatcttcctatagaatcatccttattcgttgacctagctgattctggagtgacccagagggtcatgacttgagcctaaaatccgccgcctccaccatttgtagaaaaatgtgacgaactcgtgagctctgtacagtgaccggtgactctttctggcatgcggagagacggacggacgcagagagaagggctgagtaataagccactggccagacagctctggcggctctgaggtgcagtggatgattattaatccgggaccggccgcccctccgccccgaagtggaaaggctggtgtgcccctcgttgaccaagaatctattgcatcatcggagaatatggagcttcatcgaatcaccggcagtaagcgaaggagaatgtgaagccaggggtgtatagccgtcggcgaaatagcatgccattaacctaggtacagaagtccaattgcttccgatctggtaaaagattcacgagatagtaccttctccgaagtaggtagagcgagtacccggcgcgtaagctccctaattggcgaattcccatccggcatctgtagggcgtccaaatatcgtgcctctcctgctttgccaggtgtatgaaaccggaaaggccgctcaggagctggccagcggcgcagaccgggaacacaagctggcagtcgacccatccggtgctctgcactcgacctgctgaggtccctcagtccctggtaggcagctttgccccgtctgtccgcccggtgtgtcggcggggttgacaaggtcgttgcgtcagtccaacatttgttgccatattttcctgctttccccaccagctgctcttttcttttctctttcttttcccatcttcagtatattcatcttcccatatgcatccaagaacctttatttcccctaagtaagtactttgctacatccatactccatccttcccatcccttattcctttgaacctttcagttcgagctttcccacttcatcgcagcttgactaacagctaccccgcttgagcagacatcaccatggccgttgcggactgggaggaggcgcgcggccgcatgctcctggatcccaccgttgtcaatctaaacacggggtcgggaggcccgctccccaggtccgccttcgagagggtcacaggtttccgtgcccacctggccgcggagccgatggacttcctgcttcgcgaggtgcctgctcttctctggcaggccagggagagcctcgcccgcctgatcggtggcgatcccttgcggctcgccctggcgaccaatgtcacggcagccgtgaatctggtcgccagttcgctgcgtctcgaggcaccgggtgagattcttctgtcggacgacgaatacacacccatgagatggtgctgggagcgcgtggcccgtaggcatggcttggagctccgcacattccgcctgccagagctgccaagcgatccggctgaaatcactgcagccgcagttgctgcaatgggaccgcggacgcgactctttttcttctcccacgtcgtttcgaccacgggtctcatactccccgctgcggagctctgcgaagaggcccgagcccgtggcatcacgacggtcgtcgatggcgcccatgcccctggttttctggatctcgacctcagccgtatcccgtgcgacttttacgccggttccggtcataagtggctcctggcacccactggcgttggcttcctccacttggcgccgggccgcctagaggaactcgagcctacacaggtctcatgggcctacgagcctccagagggctcgggccctccggcggcgcgagaccggtttgggagtaccccgggcctgcggaggctcgagtgcgagggcacgcgagatatctgcccctggctcgccacccccgaaagtatcgacttccaagcagagctaggtcccggggctatccgtgcgcgtcgtcgcgagctgaccgaccatgcgcggcgcctgctcgccgaccgtcctgggaggaccctccttactcctgactcgccggagctctcaggcggaatggttgcttacaggttgccacccggcaccgacgcagccgagctgcgccgtggcctgtgggagcgatttcgcatcgaggccgccgtcgccgaacagccgccgggccccgtgctacgcatctccgcgaatttctataccaccgaggaggagattgatcgactcgccgacgccctcgacgcccttacgggagagtccggccagtcggcggctcggccaagactctaatgaaagcttatcgataccgtcgacctcgagacttaacgttactgaaatcatcaaacagcttgacgaatctggatataagatcgttggtgtcgatgtcagctccggagttgagacaaatggtgttcaggatctcgataagatacgttcatttgtccaagcagcaaagagtgccttctagtgatttaatagctccatgtcaacaagaataaaacgcgttttcgggtttacctcttccagatacagctcatctgcaatgcattaatgcattgactgcaacctagtaacgcctttcaggctccggcgaagagaagaatagcttagcagagctattttcattttcgggagacgagatcaagcagatcaacggtcgtcaagagacctacgagactgaggaatccgctcttggctccacgcgactatatatttgtctctaattgtactttgacatgctcctcttctttactctgatagcttgactatgaaaattccgtcaccagcccctgggttcgcaaagataattgcatgtttcttccttgaactctcaagcctacaggacacacattcatcgtaggtataaacctcgaaatcagttcctactaagatggtatacaatagtaaccatgcatggttgcctagtgaatgctccgtaacacccaatacgccggccgaaacttttttacaactctcctatgagtcgtttacccagaatgcacaggtacacttgtttagaggtaatccttctttctagaagtcctcgtgtactgtgtaagcgcccactccacatctccactcgatggtacccaattcgccctatagtgagtcgtattaaaaccccgggtacgtaaattaaccctcactaaagggaacaaaagctgggcaaagcttgaggccggacaaattcagcctgcaggctaaagtttctattacatgatatttgtcgtggacaagggcgtctggggtaaaaaggaatgtgggcagagagctctcggcttaaagaccggcttcggagttccagacccactcgaactgaaaacgatgattagagataagtagatctatttggacagtataagaatcctagtcggctagtatttctccacttttactttaaaattccccagagtaagggggcaggttcgtcgtcacgggtagcctcgtctcgaggcatcgcggatagcattatcttggggtatcacgagtaacttcatcgtggcattatcgataggtactgtaagtactgtaggaacttatccgggcatggatatgtataggtacatacgatgcactaaaagtggagaaatactagccgagtagagatcttataccatccgaatagatttactccttataatcaaggggcaacaatcagttgtgacgatgtcggctgtgggagtgcagtttaggggtcatcaaagcacaggaaaacgtgttgtatggatgcctatcgtcttgactattagaaaggaagaggggaaaaaccctcatcaggagcgattgtaagttcggccatagtaatgatattggccattaatggacgtgtgtatgtatacatacacggttcatttgccgcattcggaccaaaaccgctgctgccgcagacacagtgcttccatggcctcgaacaaccggttattcttctcttccatgtcctcgggacgaaggaaatttcggagccctaacagccgtaccggacttgcgttaacatggttgcgaagaactaaagactgatggggtcatgattggcagtgttgacacttcatgtcttgaacctagctagcagaaaaatgaatgctctatgtgacactggtagatctcaacgcatcatgttccacctttagtgtaaacacggcaagctgtccgcaacgtcggtaccaacgtttgaacacacaaccttctgccactccaggagtttagcccacggcttactggatgaaacgtaatctcccgctaccccctcaattccattggggtctagagtagtcggaagaacggctgtcgccttgcgctgcggttaaagcacccaccgtggtggctactgcttctcgggaggagaaatcctgggtactcgagcacttgcgctaggggatgaaacatccatggcatattggcgaaagcaatgcgccatgttcggcgcggcacatgacactcttgagaagccgtattcttcgcaaactttcctatttacattcagcctctaactataacacgatcggaaatgcctgaacgagcccgccctcatgtgcctagcgtcaaacaacgccaagcacacaacgcctcctgctattcttccctcttctcactgccatcactgggcgcaagctgcaatgtccttctcgaattcaagcgggcaaatcaagattgggaaaatgcgccatcttggtttggatcttgatgtctatccgcatcaaggtcttggtttggtcgtttatttagtagcaaaggcaaatcaaaacgtgcgcgccaagtgccagggtccagactccagactggagcatttagcctgaatatcgtctctagaatctggtgctattattcaggatatagtaactatgatctactcgggccatgttcggctcctccgcacggccaagttgtctgccggcgtctggaccggactcatggcttggcttctccagggatagcatggcattggcaaaactctccgccacgattcgagcatagctaccgcagccacgcggcattgtttccagattgagatatgtcactattagccggaatgcaaacatcgagctgacctgcgcaacatctccatgagttccgaagtcgacctccgaagcaatattggtctagtattacggatgatatagtggtccccggacccaatgagccgtgtgttttttaccgcctttgctctgaggattaacaagattcgtgcaattggggactgtgcggagtaactgggctggtttactgctttgccgacgaaagaaacgtataaacagccgactcgtccactgccactcgggacgatctcccaacccagacagcttcccagaacccatcttcaacaccctgacaccatgccccagttcgacatcctatgcaagactcctccgaaggtgctcgtccgccagttcgtggagcgattcgagcgcccctcgggcgaaaagatcgccttgtgtgccgctgagcttacctacctctgctggatgatcacccacaacggcaccgccatcaagcgggctacctttatgagttacaataccatcattagcaactccctctcgtttgacatcgtcaacaagtccctgcagttcaagtacaagacccaaaaggccaccatcctcgaggcctcgctgaagaagctgatccccgcatgggaattcactatcatcccctactatggtcagaagcatcagtctgacatcaccgacattgtaagcagtctccagctccagtttgagtcctccgaggaggccgataaaggcaactcccactccaagaagatgctcaaggctttgctgagtgaaggcgagtccatctgggaaataaccgaaaagatcttgaacagtttcgagtacaccagccgcttcacgaagaccaagacgctgtaccagttcctgttcctcgccacattcatcaattgcggacgcttcagtgatatcaagaacgtggacccgaagtcattcaagctggttcagaacaagtacctcggtgtcatcattcagtgcttggtcaccgagaccaagacatccgtcagccgtcacatctacttcttttccgcaagagggcgtatcgaccccctagtgtacctagacgaattcctgcgcaactcggagcccgtcctaaagcgcgtcaaccgtaccggcaactctagcagcaacaagcaggagtaccagctcttgaaggataacctcgtccgatcatacaacaaggcgctcaagaagaacgctccatacagcatctttgctatcaagaatgggccaaagtcacacatcggccgccacctcatgacctcgtttctgtcgatgaagggcctcactgagcttaccaacgttgttggcaactggtccgataagcgcgccagcgccgtggcgcggacgacttacactcatcagatcacagctatccctgaccactacttcgccttggtcagtcgctattacgcctacgacccaattagtaaagagatgatcgctctcaaggacgaaaccaaccccatcgaggagtggcaacacatcgagcagcttaaaggctccgccgagggctcgatccggtaccccgcctggaacggtatcatatcgcaggaggtcttggattacctgagcagttatatcaatcgccgcatatgataaggatccacttaacgttactgaaatcatcaaacagcttgacgaatctggatataagatcgttggtgtcgatgtcagctccggagttgagacaaatggtgttcaggatctcgataagatacgttcatttgtccaagcagcaaagagtgccttctagtgatttaatagctccatgtcaacaagaataaaacgcgttttcgggtttacctcttccagatacagctcatctgcaatgcattaatgcattgactgcaacctagtaacgccttncaggctccggcgaagagaagaatagcttagcagagctattttcattttcgggagacgagatcaagcagatcaacggtcgtcaagagacctacgagactgaggaatccgctcttggctccacgcgactatatatttgtctctaattgtactttgacatgctcctcttctttactctgatagcttgactatgaaaattccgtcaccagcncctgggttcgcaaagataattgcatgtttcttccttgaactctcaagcctacaggacacacattcatcgtaggtataaacctcgaaatcanttcctactaagatggtatacaatagtaaccatgcatggttgcctagtgaatgctccgtaacacccaatacgccggccgaaacttttttacaactctcctatgagtcgtttacccagaatgcacaggtacacttgtttagaggtaatccttctttctagaagtcctcgtgtactgtgtaagcgcccactccacatctccactcgaccaattcgccctatagtgagtcgtattaagcttcctgcagttcgaagttcctattctctagaaagtataggaacttcagagcgctttccttgtatctctacacacaggctcaaatcaataagaagaacggttcgtctttttcgtttatatcttgcatcgtcccaaagctattggcgggatattctgtttgcagttggctgacttgaagtaatctctgcagatctttcgacactgaaatacgtcgagcctgctccgcttggaagcggcgaggagcctcgtcctgtcacaactaccaacatggagtacgataagggccagttccgccagctcattaagagccagttcatgggcgttggcatgatggccgtcatgcatctgtacttcaagtacaccaacgctcttctgatccagtcgatcatccgctgaaggcgctttcgaatctggttaagatccacgtcttcgggaagccagcgactggtgacctccagcgtccctttaaggctgccaacagctttctcagccagggccagcccaagaccgacaaggcctccctccagaacgccgagaagaactggaggggtggtgtcaaggaggagtaagctccttattgaagtcggaggacggagcggtgtcaagaggatattcttcgactctgtattatagataagatgatgaggaattggaggtagcatagcttcatttggatttgctttccaggctgagactctagcttggagcatagagggtcctttggctttcaatattctcaagtatctcgagtttgaacttattccctgtgaaccttttattcaccaatgagcattggaatgaacatgaatctgaggactgcaatcgccatgaggttttcgaaatacatccggatgtcgaaggcttggggcacctgcgttggttgaatttagaacgtggcactattgatcatccgatagctctgcaaagggcgttgcacaatgcaagtcaaacgttgctagcagttccaggtggaatgttatgatgagcattgtattaaatcaggagatatagcatgatctctagttagctcaccacaaaagtcagacggcgtaaccaaaagtcacacaacacaagctgtaaggatttcggcacggctacggaagacggagaagccaccttcagtggactcgagtaccatttaattctatttgtgtttgatcgagacctaatacagcccctacaacgaccatcaaagtcgtatagctaccagtgaggaagtggactcaaatcgacttcagcaacatctcctggataaactttaagcctaaactatacagaataagataggtggagagcttataccgagctcccaaatctgtccagatcatggttgaccggtgcctggatcttcctatagaatcatccttattcgttgacctagctgattctggagtgacccagagggtcatgacttgagcctaaaatccgccgcctccaccatttgtagaaaaatgtgacgaactcgtgagctctgtacagtgaccggtgactctttctggcatgcggagagacggacggacgcagagagaagggctgagtaataagccactggccagacagctctggcggctctgaggtgcagtggatgattattaatccgggaccggccgcccctccgccccgaagtggaaaggctggtgtgcccctcgttgaccaagaatctattgcatcatcggagaatatggagcttcatcgaatcaccggcagtaagcgaaggagaatgtgaagccaggggtgtatagccgtcggcgaaatagcatgccattaacctaggtacagaagtccaattgcttccgatctggtaaaagattcacgagatagtaccttctccgaagtaggtagagcgagtacccggcgcgtaagctccctaattggcccatccggcatctgtagggcgtccaaatatcgtgcctctcctgctttgcccggtgtatgaaaccggaaaggccgctcaggagctggccagcggcgcagaccgggaacacaagctggcagtcgacccatccggtgctctgcactcgacctgctgaggtccctcagtccctggtaggcagctttgccccgtctgtccgcccggtgtgtcggcggggttgacaaggtcgttgcgtcagtccaacatttgttgccatattttcctgctctccccaccagctgctcttttcttttctctttcttttcccatcttcagtatattcatcttcccatccaagaacctttatttcccctaagtaagtactttgctacatccatactccatccttcccatcccttattcctttgaacctttcagttcgagctttcccacttcatcgcagcttgactaacagctaccccgcttgagcagacatcaccatgcctgaactcaccgcgacgtctgtcgagaagtttctgatcgaaaagttcgacagcgtctccgacctgatgcagctctcggagggcgaagaatctcgtgctttcagcttcgatgtaggagggcgtggatatgtcctgcgggtaaatagctgcgccgatggtttctacaaagatcgttatgtttatcggcactttgcatcggccgcgctcccgattccggaagtgcttgacattggggaattcagcgagagcctgacctattgcatctcccgccgtgcacagggtgtcacgttgcaagacctgcctgaaaccgaactgcccgctgttctgcagccggtcgcggaggccatggatgcgatcgctgcggccgatcttagccagacgagcgggttcggcccattcggaccgcaaggaatcggtcaatacactacatggcgtgatttcatatgcgcgattgctgatccccatgtgtatcactggcaaactgtgatggacgacaccgtcagtgcgtccgtcgcgcaggctctcgatgagctgatgctttgggccgaggactgccccgaagtccggcacctcgtgcacgcggatttcggctccaacaatgtcctgacggacaatggccgcataacagcggtcattgactggagcgaggcgatgttcggggattcccaatacgaggtcgccaacatcttcttctggaggccgtggttggcttgtatggagcagcagacgcgctacttcgagcggaggcatccggagcttgcaggatcgccgcggctccgggcgtatatgctccgcattggtcttgaccaactctatcagagcttggttgacggcaatttcgatgatgcagcttgggcgcagggtcgatgcgacgcaatcgtccgatccggagccgggactgtcgggcgtacacaaatcgcccgcagaagcgcggccgtctggaccgatggctgtgtagaagtactcgccgatagtggaaaccgacgccccagcactcgtccgagggcaaaggaatagagtagatgccgaccgcgggatccacttaacgttactgaaatcatcaaacagcttgacgaatctggatataagatcgttggtgtcgatgtcagctccggagttgagacaaatggtgttcaggatctcgataagatacgttcatttgtccaagcagcaaagagtgccttctagtgatttaatagctccatgtcaacaagaataaaacgcgttttcgggtttacctcttccagatacagctcatctgcaatgcattaatgcattgactgcaacctagtaacgccttncaggctccggcgaagagaagaatagcttagcagagctattttcattttcgggagacgagatcaagcagatcaacggtcgtcaagagacctacgagactgaggaatccgctcttggctccacgcgactatatatttgtctctaattgtactttgacatgctcctcttctttactctgatagcttgactatgaaaattccgtcaccagcncctgggttcgcaaagataattgcatgtttcttccttgaactctcaagcctacaggacacacattcatcgtaggtataaacctcgaaatcanttcctactaagatggtatacaatagtaaccatgcatggttgcctagtgaatgctccgtaacacccaatacgccggccgaaacttttttacaactctcctatgagtcgtttacccagaatgcacaggtacacttgtttagaggtaatccttctttctagaagtcctcgtgtactgtgtaagcgcccactccacatctccactcgacctgcagttcgaagttcctattctctagaaagtataggaacttcagagcgctttccaattcgccctatagtgagtcgtattacgcgcgctcactggccgtcgttttacaacgtcgtgactgggaaaaccctggcgttacccaacttaatcgccttgcagcacatccccctttcgccagctggcgtaatagcgaagaggcccgcaccgatcgcccttcccaacagttgcgcagcctgaatggcgaatgggacgcgccctgtagcggcgcattaagcgcggcgggtgtggtggttacgcgcagcgtgaccgctacacttgccagcgccctagcgcccgctcctttcgctttcttcccttcctttctcgccacgttcgccggctttccccgtcaagctctaaatcgggggctccctttagggttccgatttagtgctttacggcacctcgaccccaaaaaacttgattagggtgatggttcacgtagtgggccatcgccctgatagacggtttttcgccctttgacgttggagtccacgttctttaatagtggactcttgttccaaactggaacaacactcaaccctatctcggtctattcttttgatttataagggattttgccgatttcggcctattggttaaaaaatgagctgatttaacaaaaatttaacgcgaattttaacaaaatattaacgcttacaatttag

SEQ ID NO: 23 - DNA, 2079 bp, synthetic construct
  misc_feature 1..2079: note = Nucleic acid sequence of CPC acylase
  source 1..2079: mol_type = other DNA
atggaaccgaccagcaccccgcaggctccgatcgctgcttataaaccgcgtagcaacgaaatcctgtgggatggttatggtgttccgcatatctatggtgttgacgctccgagcgctttttatggttatggctgggctcaggctcgtagccatggtgataacatcctgcgtctgtatggtgaagctcgtggtaaaggcgctgaatattggggtccggattacgaacagacgaccgtttggctgctgaccaacggtgttccggaacgtgctcagcagtggtatgctcagcagagcccggattttcgtgctaacctggatgcttttgctgctggtatcaacgcttatgctcagcagaacccggatgatatcagcccggaagttcgtcaggttctgccggttagcggtgctgatgttgttgctcatgctcatcgtctgatgaactttctgtatgttgctagcccgggtcgtaccctgggtgaaggtgatccgccggatctggctgatcagggtagcaacagctgggctgttgctccgggtaaaaccgctaacggtaacgctctgctgctgcagaaccctcatctgagctggaccaccgattattttacctattatgaagctcatctggttaccccggattttgaagtgtatggtgctacccagatcggtctgccggttatccgtgttgcttttaaccagcgtatgggtatcaccaacaccgttaacggtatggttggtgctaccaactatcgtctgaccctgcaggatggtggttatctgtatgatggtcaggttcgtccgtttgaacgtcgtcaggctagctatcgtctgcgtcaggctgatggtaccaccgttgataaaccgctggaaatccgttccagcgttcatggtccggtttttgaacgtgctgatggtaccgctgttgctgttcgtgttgctggtctggatcgtccgggtatgctggaacagacttttgatatgatcaccgctgatagctttgatgattatgaagctgctctggctcgtatgcaggttccgaccttgaacatcgtttatgctgatcgtgaaggtaccatcaactatagctttaacggtgttgctccgaaacgtgctgaaggtgacatcgctttttggcagggtctggttccgggtgatagcagccgttatctgtggaccgaaacccatccgctggatgatctgccgcgtgttaccaacccgccgggtggttttgttcagaacagcaacgatccgccgtggaccccgacctggccggttacctataccccgaaagattttccgagctatctggctccgcagaccccgcatagcctgcgtgctcagcagagcgttcgtctgatgagcgaaaacgatgatctgaccctggaacgttttatggctctgcagctgagccatcgtgctgttatggctgatcgtaccctgccggatctgatcccggctgctctgatcgatccggatccggaagttcaggctgctgctcgtctgctggctgcgtgggatcgtgaatttaccagcgatagccgtgctgctctgctgtttgaagaatgggctcgtctgtttgctggtcagaactttgctggtcaggctggctttgctaccccgtggagcctggataaaccggttagcaccccgtatggtctgcgtgatccgaaagctgctgttgatcagctgcgtaccgctatcgctaacaccaaacgtaaatatggtgctatcgatcgtccgtttggtgatgctagccgtatgatcctgaacgatgttaacgttccgggtgctgctggttatggtaacctgggtagctttcgtgtttttacctggagcgatccggatgaaaacggtgtgcgtaccccggttcatggtgaaacctgggttgctatgatcgaatttagcaccccggttcgtgcttatggtctgatgagctatggtaacagccgtcagccgggtaccacccattatagcgatcagatcgaacgtgttagccgtgctgattttcgtgaactgctgctgcgtcgtgaacaggttgaagctgctgttcaggaacgtaccccgtttaactttaaaccgtga